European Patent Application EP 4 428 149 A1, published September 11, 2024. Title: Antibody Specific for Resistin and Uses Thereof. Applicant: SEOUL NATIONAL UNIVERSITY HOSPITAL. The sequence listing filed with the application follows.

SEQUENCE LISTING (63 sequences)

SEQ ID NO: 1 - protein, 5 aa, synthetic construct
SYAIS

SEQ ID NO: 2 - protein, 17 aa, synthetic construct
GIIPIFGAADYAQKFKG

SEQ ID NO: 3 - protein, 10 aa, synthetic construct
GPDYYGSFDP

SEQ ID NO: 4 - protein, 17 aa, synthetic construct
KSSQSVLYSSNNKNYLA

SEQ ID NO: 5 - protein, 12 aa, synthetic construct
RASQSVRGSYLA

SEQ ID NO: 6 - protein, 14 aa, synthetic construct
TGTSSDIGRYNRVS

SEQ ID NO: 7 - protein, 11 aa, synthetic construct
RASQSIGTYLN

SEQ ID NO: 8 - protein, 11 aa, synthetic construct
QASQHVSSYLN

SEQ ID NO: 9 - protein, 11 aa, synthetic construct
RTSQTITNYLN

SEQ ID NO: 10 - protein, 14 aa, synthetic construct
TGSSSDVGGYNYVT

SEQ ID NO: 11 - protein, 11 aa, synthetic construct
RASQYIGTYLA

SEQ ID NO: 12 - protein, 7 aa, synthetic construct
WASTRES

SEQ ID NO: 13 - protein, 7 aa, synthetic construct
GTSSRAP

SEQ ID NO: 14 - protein, 7 aa, synthetic construct
DVSNRPS

SEQ ID NO: 15 - protein, 7 aa, synthetic construct
DASSLED

SEQ ID NO: 16 - protein, 7 aa, synthetic construct
AASNLQS

SEQ ID NO: 17 - protein, 7 aa, synthetic construct
DASNLET

SEQ ID NO: 18 - protein, 7 aa, synthetic construct
DVTKRPS

SEQ ID NO: 19 - protein, 7 aa, synthetic construct
GASILQN

SEQ ID NO: 20 - protein, 8 aa, synthetic construct
QQYYSEPL

SEQ ID NO: 21 - protein, 9 aa, synthetic construct
QQRGDWLYT

SEQ ID NO: 22 - protein, 10 aa, synthetic construct
SAYTRSSTWV

SEQ ID NO: 23 - protein, 10 aa, synthetic construct
QQSYTMPLYT

SEQ ID NO: 24 - protein, 11 aa, synthetic construct
QQYDSYSSVYT

SEQ ID NO: 25 - protein, 9 aa, synthetic construct
QQSYNPGYT

SEQ ID NO: 26 - protein, 10 aa, synthetic construct
SSYSSSTFYV

SEQ ID NO: 27 - protein, 9 aa, synthetic construct
QQADSFPLT

SEQ ID NO: 28 - protein, 119 aa, synthetic construct
QVQLVQSGAEGRKPGSSVKVSCKVSGDTFSSYAISWVRQAPGQGLEWMGGIIPIFGAADYAQKFKGRVTISADESTSTAYMELSSLRSEDTAVYYCAKGPDYYGSFDPWGQGTLITVSS

SEQ ID NO: 29 - protein, 330 aa, synthetic construct
ASTKGPSVFPLAPSSKSTSGGTAALGCLVKDYFPEPVTVSWNSGALTSGVHTFPAVLQSSGLYSLSSVVTVPSSSLGTQTYICNVNHKPSNTKVDKKVEPKSCDKTHTCPPCPAPELLGGPSVFLFPPKPKDTLMISRTPEVTCVVVDVSHEDPEVKFNWYVDGVEVHNAKTKPREEQYNSTYRVVSVLTVLHQDWLNGKEYKCKVSNKALPAPIEKTISKAKGQPREPQVYTLPPSREEMTKNQVSLTCLVKGFYPSDIAVEWESNGQPENNYKTTPPVLDSDGSFFLYSKLTVDKSRWQQGNVFSCSVMHEALHNHYTQKSLSLSPGK

SEQ ID NO: 30 - DNA, 357 bp, synthetic construct
  source 1..357: mol_type = other DNA
caggtgcagctggtgcagtctggggctgaggggaggaagcctgggtcctcggtgaaggtctcctgcaaggtttctggagacaccttcagcagttatgctatcagctgggtgcgacaggcccctggacaagggcttgagtggatgggagggatcatccctatctttggtgcagcagactacgcacagaagttcaagggcagagtcacgattagtgcggacgaatccacgagcacagcctacatggagctgagcagcctgagatctgaggacacggccgtgtattactgtgcgaaaggaccggattattatggttcgtttgacccctggggccagggaaccctgatcaccgtctcctca

SEQ ID NO: 31 - DNA, 990 bp, synthetic construct
  source 1..990: mol_type = other DNA
gctagcaccaagggcccatcggtcttccccctggcaccctcctccaagagcacctctgggggcacagcggccctgggctgcctggtcaaggactacttccccgaaccggtgacggtgtcgtggaactcaggcgccctgaccagcggcgtgcacaccttcccggctgtcctacagtcctcaggactctactccctcagcagcgtggtgaccgtgccctccagcagcctgggcacccagacctacatctgcaacgtgaatcacaagcccagcaacaccaaggtggacaagaaagttgagcccaaatcttgtgacaaaactcacacatgcccaccgtgcccagcacctgaactcctggggggaccgtcagtcttcctcttccccccaaaacccaaggacaccctcatgatctcccggacccctgaggtcacatgcgtggtggtggacgtgagccacgaagaccctgaggtcaagttcaactggtacgtggacggcgtggaggtgcataatgccaagacaaagccgcgggaggagcagtacaacagcacgtaccgtgtggtcagcgtcctcaccgtcctgcaccaggactggctgaatggcaaggagtacaagtgcaaggtctccaacaaagccctcccagcccccatcgagaaaaccatctccaaagccaaagggcagccccgagaaccacaggtgtacaccctgcccccatcccgggaggagatgaccaagaaccaggtcagcctgacctgcctggtcaaaggcttctatcccagcgacatcgccgtggagtgggagagcaatgggcagccggagaacaactacaagaccacgcctcccgtgctggactccgacggctccttcttcctctacagcaagctcaccgtggacaagagcaggtggcagcaggggaacgtcttctcatgctccgtgatgcatgaggctctgcacaaccactacacgcagaagagcctctccctgtctccgggtaaa

SEQ ID NO: 32 - protein, 112 aa, synthetic construct
DIQMTQSPDSLAVSLGERATINCKSSQSVLYSSNNKNYLAWYQHKPGQPPRLLIYWASTRESGVPDRFSGSGSGTDFTLTINGLQAEDVAVYYCQQYYSEPLFGPGTKVDIK

SEQ ID NO: 33 - protein, 107 aa, synthetic construct
RSVAAPSVFIFPPSDEQLKSGTASVVCLLNNFYPREAKVQWKVDNALQSGNSQESVTEQDSKDSTYSLSSTLTLSKADYEKHKVYACEVTHQGLSSPVTKSFNRGEC

SEQ ID NO: 34 - protein, 108 aa, synthetic construct
DIQMTQSPGTLSLSAGERATLSCRASQSVRGSYLAWYQQKPGQAPRLLIYGTSSRAPGIPDRFSGSGSGTDFTLTISSLEPEDFAVYYCQQRGDWLYTFGQGTKVEIK

SEQ ID NO: 35 - protein, 107 aa, synthetic construct; identical to SEQ ID NO: 33

SEQ ID NO: 36 - protein, 110 aa, synthetic construct
QSALTQPASVSGSPGQSVTISCTGTSSDIGRYNRVSWYQHHPGKAPKLIIYDVSNRPSGVSNRFSGSKSGNTASLTISGLQAGDESDYYCSAYTRSSTWVFGGGTKLTVL

SEQ ID NO: 37 - protein, 107 aa, synthetic construct; identical to SEQ ID NO: 33

SEQ ID NO: 38 - protein, 108 aa, synthetic construct
DIQMTQSPSSLSASVGDRVTITCRASQSIGTYLNWYQQKPGKAPKLLIYDASSLEDGVPSRFSGSGSGTDFTLTISSLQPEDSATYYCQQSYTMPLYTFGQGTKLEIK

SEQ ID NO: 39 - protein, 107 aa, synthetic construct; identical to SEQ ID NO: 33

SEQ ID NO: 40 - protein, 109 aa, synthetic construct
DIQMTQSPSSLSASVGDRVTITCQASQHVSSYLNWYQQKPGKAPKLLIYAASNLQSGVPSRFSGSGSGTDFTLTISSLQPDDFATYYCQQYDSYSSVYTFGPGTKLDIK

SEQ ID NO: 41 - protein, 107 aa, synthetic construct; identical to SEQ ID NO: 33

SEQ ID NO: 42 - protein, 107 aa, synthetic construct
DIQMTQSPSSLSASVGDRVTITCRTSQTITNYLNWYQQKPGRAPKLLIFDASNLETGVPSRFSGSGSGTDFTLTISSLQPEDFATYFCQQSYNPGYTFGQGTKLEIK

SEQ ID NO: 43 - protein, 107 aa, synthetic construct; identical to SEQ ID NO: 33

SEQ ID NO: 44 - protein, 110 aa, synthetic construct
NFMLTQPASVSGSPGQSITISCTGSSSDVGGYNYVTWYQQHPGKAPQLIIYDVTKRPSGVSNRFSGSKSGNSASLTISGLQAEDEADYYCSSYSSSTFYVFGTGTKVTVL

SEQ ID NO: 45 - protein, 107 aa, synthetic construct; identical to SEQ ID NO: 33

SEQ ID NO: 46 - protein, 107 aa, synthetic construct
DIQMTQSPSFLSASVGDRVTITCRASQYIGTYLAWYQQQPGKAPKLLIYGASILQNGVPSRFSGSASGTEFTLTISSLQPEDFATYYCQQADSFPLTFGGGTKVDIK

SEQ ID NO: 47 - protein, 107 aa, synthetic construct; identical to SEQ ID NO: 33

SEQ ID NO: 48 - DNA, 336 bp, synthetic construct
  source 1..336: mol_type = other DNA
gacatccagatgacccagtctccagactccctggctgtgtctctgggcgagagggccaccatcaactgcaagtccagccagagcgttttatacagctccaacaataagaactacttagcttggtaccaacacaaaccgggacaacctcctaggttgctcatttactgggcatccacccgggaatccggggtccccgatcgattcagtggcagcgggtctgggacagatttcactctcaccatcaacggcctgcaggctgaagatgtggcagtttattactgtcagcagtattatagtgagccccttttcggccctgggaccaaagtggatatcaaa

SEQ ID NO: 49 - DNA, 321 bp, synthetic construct
  source 1..321: mol_type = other DNA
agatctgtggctgcaccatctgtcttcatcttcccgccatctgatgagcagttgaaatctggaactgcctctgttgtgtgcctgctgaataacttctatcccagagaggccaaagtacagtggaaggtggataacgccctccaatcgggtaactcccaggagagtgtcacagagcaggacagcaaggacagcacctacagcctcagcagcaccctgacgctgagcaaagcagactacgagaaacacaaagtctacgcctgcgaagtcacccatcagggcctgagctcgcccgtcacaaagagcttcaacaggggagagtgt

SEQ ID NO: 50 - DNA, 324 bp, synthetic construct
  source 1..324: mol_type = other DNA
gacatccagatgacccagtctccaggcaccctgtctttgtctgcaggagaaagagccaccctctcctgcagggccagtcagagtgttaggggcagttacttagcctggtaccagcagaaacctggccaggctcccaggctcctcatctatggtacatccagcagggcccctggcatcccagacaggttcagtggcagtgggtctgggacagacttcactctcaccatcagcagcctagagcctgaagattttgcagtttattactgtcagcagcgtggcgactggctttacacttttggccaagggaccaaggtggagatcaaa

SEQ ID NO: 51 - DNA, 321 bp, synthetic construct; identical to SEQ ID NO: 49
  source 1..321: mol_type = other DNA

SEQ ID NO: 52 - DNA, 330 bp, synthetic construct
  source 1..330: mol_type = other DNA
cagtctgccctgactcagcctgcctccgtgtctgggtctcctggacagtcggtcaccatctcctgcactggaaccagcagtgacattggtcgttataaccgtgtctcctggtaccaacaccaccccggcaaggcccccaaactcatcatttatgatgtcagtaatcggccctcaggggtctctaatcgcttctccggttccaagtctggcaacacggcctccctgaccatctctgggctccaggctggggacgagtctgattattactgcagcgcatatacaaggagcagcacttgggtgttcggcggagggaccaagctgaccgtccta

SEQ ID NO: 53 - DNA, 321 bp, synthetic construct; identical to SEQ ID NO: 49
  source 1..321: mol_type = other DNA

SEQ ID NO: 54 - DNA, 324 bp, synthetic construct
  source 1..324: mol_type = other DNA
gacatccagatgacccagtctccatcctccctgtctgcttctgtaggagacagagtcaccatcacttgccgggcaagtcagagcattggcacctatttaaattggtatcagcagaaaccggggaaagctcctaagctcctgatctatgatgcctccagtttggaagatggggtcccatcaaggttcagcggcagtggatctgggacagatttcactctcaccatcagcagcctgcagcctgaagattctgcaacttactactgtcaacagagttacactatgcccctttacacttttggccaggggaccaagctggaaatcaaa

SEQ ID NO: 55 - DNA, 321 bp, synthetic construct; identical to SEQ ID NO: 49
  source 1..321: mol_type = other DNA

SEQ ID NO: 56 - DNA, 327 bp, synthetic construct
  source 1..327: mol_type = other DNA
gacatccagatgacccagtctccatcctccctgtctgcatctgtaggagacagagtcaccatcacttgccaggcgagtcaacacgttagcagctatttaaattggtatcagcagaaaccagggaaagcccctaagctcctgatctatgctgcatccaatttgcaaagtggggtcccatcaaggttcagcggcagtggatctgggacagatttcactctcaccatcagcagtctgcaacctgatgattttgcaacttattactgccaacagtatgatagttattcttcggtgtacacctttggcccggggaccaagctggatatcaaa

SEQ ID NO: 57 - DNA, 321 bp, synthetic construct; identical to SEQ ID NO: 49
  source 1..321: mol_type = other DNA

SEQ ID NO: 58 - DNA, 321 bp, synthetic construct
  source 1..321: mol_type = other DNA
gacatccagatgacccagtctccatcctccctgtctgcatctgtaggagacagagtcaccataacttgccggacaagtcagaccataaccaactatttaaattggtatcagcagaaaccagggagagcccctaagctcctgatcttcgatgcatccaatttggaaacaggggtcccatcaagattcagcggcagtggatctgggacagatttcactctcaccatcagcagtctgcaacctgaagattttgcaacttacttctgtcaacagagttacaatcccgggtacacctttggccaggggaccaagctggagatcaaa

SEQ ID NO: 59 - DNA, 321 bp, synthetic construct; identical to SEQ ID NO: 49
  source 1..321: mol_type = other DNA

SEQ ID NO: 60 - DNA, 330 bp, synthetic construct
  source 1..330: mol_type = other DNA
aattttatgctgactcagcccgcctccgtgtctgggtcccctggacagtcgatcaccatctcctgcactggaagcagcagcgacgttggtggttataactatgtcacctggtaccaacagcacccaggcaaagccccccaactcatcatttatgatgtcactaagcggccctcaggggtttctaatcgcttctccggctccaagtctggcaactcggcctccctgaccatctctggactccaggctgaggacgaggctgattattactgcagctcatacagcagcagcactttttacgtcttcggaactgggaccaaggtcaccgtccta

SEQ ID NO: 61 - DNA, 321 bp, synthetic construct; identical to SEQ ID NO: 49
  source 1..321: mol_type = other DNA

SEQ ID NO: 62 - DNA, 321 bp, synthetic construct
  source 1..321: mol_type = other DNA
gacatccagatgacccagtctccatccttcctgtctgcatctgtaggagacagagtcaccatcacttgtcgggccagtcagtacattggtacttatttagcctggtatcagcaacaaccagggaaagcccctaagctcctgatttatggtgcatccattttgcaaaatggggtcccatcaaggttcagcggcagtgcatctgggacagaattcactctcacaatcagcagcctgcagcctgaagattttgcaacttattattgtcaacaggctgacagtttcccgctcactttcggcggagggaccaaggtggatatcaaa

SEQ ID NO: 63 - DNA, 321 bp, synthetic construct; identical to SEQ ID NO: 49
  source 1..321: mol_type = other DNA